European Patent Specification EP 2 945 701 B1, published April 5, 2023. Title: METHODS OF TREATING DISEASES ASSOCIATED WITH HIGH-FAT DIET AND VITAMIN A DEFICIENCIES USING RETINOIC ACID RECEPTOR AGONISTS. Applicant: Cornell University. Application PCT/US14/999999. The sequence listing filed with the application follows.

SEQUENCE LISTING (38 sequences)

SEQ ID NO: 1 - DNA, 22 bp, Artificial Sequence
  mIns1 primer
tagtgaccagctataatcagag

SEQ ID NO: 2 - DNA, 20 bp, Artificial Sequence
  mIns1 primer
acgccaaggtctgaaggtcc

SEQ ID NO: 3 - DNA, 19 bp, Artificial Sequence
  mGcg primer
ccgccgtgcccaagatttt

SEQ ID NO: 4 - DNA, 17 bp, Artificial Sequence
  mGcg primer
cctgcggccgagttcct

SEQ ID NO: 5 - DNA, 20 bp, Artificial Sequence
  mSst* primer
gagcccaaccagacagagaa

SEQ ID NO: 6 - DNA, 20 bp, Artificial Sequence
  mSst* primer
gaagttcttgcagccagctt

SEQ ID NO: 7 - DNA, 24 bp, Artificial Sequence
  mNgn3* primer
ctgcgcatagcggaccacagcttc

SEQ ID NO: 8 - DNA, 26 bp, Artificial Sequence
  mNgn3* primer
cttcacaagaagtctgagaacaccag

SEQ ID NO: 9 - DNA, 20 bp, Artificial Sequence
  mRAR  primer
gatcctggatttctacaccg

SEQ ID NO: 10 - DNA, 19 bp, Artificial Sequence
  mRAR  primer
cactgacgccatagtggta

SEQ ID NO: 11 - DNA, 23 bp, Artificial Sequence
  mNanog primer
aaaggatgaagtgcaagcggtgg

SEQ ID NO: 12 - DNA, 21 bp, Artificial Sequence
  mNanog primer
ctggctttgccctgactttaa

SEQ ID NO: 13 - DNA, 24 bp, Artificial Sequence
  mRex1 primer
gaaagcaggatcgcctcactgtgc

SEQ ID NO: 14 - DNA, 23 bp, Artificial Sequence
  mRex1 primer
cgataagacaccacagtacacac

SEQ ID NO: 15 - DNA, 24 bp, Artificial Sequence
  mCyp26a1 primer
gaaacattgcagatggtgcttcag

SEQ ID NO: 16 - DNA, 23 bp, Artificial Sequence
  mCyp26a1 primer
cggctgaaggcctgcataatcac

SEQ ID NO: 17 - DNA, 23 bp, Artificial Sequence
  mPax-6 primer
gcaacccccagtccccagtcaga

SEQ ID NO: 18 - DNA, 24 bp, Artificial Sequence
  mPax-6 primer
agtccattcccgggctccagttca

SEQ ID NO: 19 - DNA, 18 bp, Artificial Sequence
  mIsl-1* primer
cccgggggccactatttg

SEQ ID NO: 20 - DNA, 17 bp, Artificial Sequence
  mIsl-1* primer
cgggcacgcatcacgaa

SEQ ID NO: 21 - DNA, 20 bp, Artificial Sequence
  mIapp* primer
tgggctgtagttcctgaagc

SEQ ID NO: 22 - DNA, 20 bp, Artificial Sequence
  mIapp* primer
gcacttccgtttgtccatct

SEQ ID NO: 23 - DNA, 20 bp, Artificial Sequence
  HPRT1 primer
tgctcgagatgtgatgaagg

SEQ ID NO: 24 - DNA, 20 bp, Artificial Sequence
  HPRT1 primer
tcccctgttgactggtcatt

SEQ ID NO: 25 - DNA, 20 bp, Artificial Sequence
  RAR-beta-2 primer
tggcattgtttgcacgctga

SEQ ID NO: 26 - DNA, 22 bp, Artificial Sequence
  RAR-beta-2 primer
cccccctttggcaaagaataga

SEQ ID NO: 27 - DNA, 23 bp, Artificial Sequence
  CYP26A1 RAR-beta-2 primer
ctttataaggccgcccaggttac

SEQ ID NO: 28 - DNA, 22 bp, Artificial Sequence
  CYP26A1 RAR-beta-2 primer
cccgatccgcaattaaagatga

SEQ ID NO: 29 - DNA, 21 bp, Artificial Sequence
  LRAT primer
tctggcatctctcctacgctg

SEQ ID NO: 30 - DNA, 24 bp, Artificial Sequence
  LRAT primer
gttccaagtccttcagtctcttgc

SEQ ID NO: 31 - DNA, 22 bp, Artificial Sequence
  INS2 primer
tgtggggagcgtggcttcttct

SEQ ID NO: 32 - DNA, 22 bp, Artificial Sequence
  INS2 primer
cagctccagttgtgccacttgt

SEQ ID NO: 33 - DNA, 19 bp, Artificial Sequence
  HPRT primer
tgctcgagtgtgatgaagg

SEQ ID NO: 34 - DNA, 19 bp, Artificial Sequence
  HPRT primer
tccctgttgactggtcatt

SEQ ID NO: 35 - DNA, 19 bp, Artificial Sequence
  TNF-alpha primer
cctgtagcccacgtcgtag

SEQ ID NO: 36 - DNA, 22 bp, Artificial Sequence
  TNF-alpha primer
gggagtagacaaggtacaaccc

SEQ ID NO: 37 - DNA, 23 bp, Artificial Sequence
  MCP1 primer
ttaaaaacctggatcggaaccaa

SEQ ID NO: 38 - DNA, 23 bp, Artificial Sequence
  MCP1 primer
gcattagcttcagatttacgggt